European Patent Specification EP 3 388 075 B1, published May 24, 2023. Title: Novel peptides and combination of peptides for use in immunotherapy against various tumors. Applicant: Immatics Biotechnologies GmbH. The sequence listing filed with the application follows.

SEQUENCE LISTING (290 sequences)

SEQ ID NO: 1 - protein, 9 aa, Homo sapiens
KLQEKIQEL

SEQ ID NO: 2 - protein, 10 aa, Homo sapiens
SVLEKEIYSI

SEQ ID NO: 3 - protein, 11 aa, Homo sapiens
RVIDDSLVVGV

SEQ ID NO: 4 - protein, 9 aa, Homo sapiens
VLFGELPAL

SEQ ID NO: 5 - protein, 9 aa, Homo sapiens
GLVDIMVHL

SEQ ID NO: 6 - protein, 9 aa, Homo sapiens
FLNAIETAL

SEQ ID NO: 7 - protein, 9 aa, Homo sapiens
ALLQALMEL

SEQ ID NO: 8 - protein, 9 aa, Homo sapiens
ALSSSQAEV

SEQ ID NO: 9 - protein, 11 aa, Homo sapiens
SLITGQDLLSV

SEQ ID NO: 10 - protein, 9 aa, Homo sapiens
QLIEKNWLL

SEQ ID NO: 11 - protein, 9 aa, Homo sapiens
LLDPKTIFL

SEQ ID NO: 12 - protein, 10 aa, Homo sapiens
RLLDPKTIFL

SEQ ID NO: 13 - protein, 9 aa, Homo sapiens
RLHDENILL

SEQ ID NO: 14 - protein, 9 aa, Homo sapiens
YTFSGDVQL

SEQ ID NO: 15 - protein, 9 aa, Homo sapiens
GLPSATTTV

SEQ ID NO: 16 - protein, 9 aa, Homo sapiens
SLADLSLLL

SEQ ID NO: 17 - protein, 11 aa, Homo sapiens
GLLPSAESIKL

SEQ ID NO: 18 - protein, 9 aa, Homo sapiens
KTASINQNV

SEQ ID NO: 19 - protein, 10 aa, Homo sapiens
KVFELDLVTL

SEQ ID NO: 20 - protein, 10 aa, Homo sapiens
ALVEKGEFAL

SEQ ID NO: 21 - protein, 9 aa, Homo sapiens
YLMDDFSSL

SEQ ID NO: 22 - protein, 9 aa, Homo sapiens
LMYPYIYHV

SEQ ID NO: 23 - protein, 9 aa, Homo sapiens
ALLSPLSLA

SEQ ID NO: 24 - protein, 9 aa, Homo sapiens
KVWSDVTPL

SEQ ID NO: 25 - protein, 11 aa, Homo sapiens
LLWGHPRVALA

SEQ ID NO: 26 - protein, 9 aa, Homo sapiens
VLDGKVAVV

SEQ ID NO: 27 - protein, 9 aa, Homo sapiens
GLLGKVTSV

SEQ ID NO: 28 - protein, 11 aa, Homo sapiens
IKVTDPQLLEL

SEQ ID NO: 29 - protein, 9 aa, Homo sapiens
KMISAIPTL

SEQ ID NO: 30 - protein, 9 aa, Homo sapiens
IITEVITRL

SEQ ID NO: 31 - protein, 11 aa, Homo sapiens
GLLETTGLLAT

SEQ ID NO: 32 - protein, 9 aa, Homo sapiens
VVMVLVLML

SEQ ID NO: 33 - protein, 9 aa, Homo sapiens
TLDRNSLYV

SEQ ID NO: 34 - protein, 9 aa, Homo sapiens
TLNTLDINL

SEQ ID NO: 35 - protein, 9 aa, Homo sapiens
VIIKGLEEI

SEQ ID NO: 36 - protein, 9 aa, Homo sapiens
TVLQELINV

SEQ ID NO: 37 - protein, 9 aa, Homo sapiens
QIVELIEKI

SEQ ID NO: 38 - protein, 9 aa, Homo sapiens
VLQQESNFL

SEQ ID NO: 39 - protein, 9 aa, Homo sapiens
YLEDGFAYV

SEQ ID NO: 40 - protein, 11 aa, Homo sapiens
KIWEELSVLEV

SEQ ID NO: 41 - protein, 9 aa, Homo sapiens
IVTEIISEI

SEQ ID NO: 42 - protein, 9 aa, Homo sapiens
KQMSISTGL

SEQ ID NO: 43 - protein, 9 aa, Homo sapiens
LLIPFTIFM

SEQ ID NO: 44 - protein, 9 aa, Homo sapiens
AVFNLVHVV

SEQ ID NO: 45 - protein, 9 aa, Homo sapiens
FLPVSVVYV

SEQ ID NO: 46 - protein, 10 aa, Homo sapiens
ISLDEVAVSL

SEQ ID NO: 47 - protein, 9 aa, Homo sapiens
GLNGFNVLL

SEQ ID NO: 48 - protein, 10 aa, Homo sapiens
KISDFGLATV

SEQ ID NO: 49 - protein, 11 aa, Homo sapiens
KLIGNIHGNEV

SEQ ID NO: 50 - protein, 9 aa, Homo sapiens
ILLSVLHQL

SEQ ID NO: 51 - protein, 9 aa, Homo sapiens
LDSEALLTL

SEQ ID NO: 52 - protein, 9 aa, Homo sapiens
TIGIPFPNV

SEQ ID NO: 53 - protein, 9 aa, Homo sapiens
AQHLSTLLL

SEQ ID NO: 54 - protein, 9 aa, Homo sapiens
YLVPGLVAA

SEQ ID NO: 55 - protein, 9 aa, Homo sapiens
HLFDKIIKI

SEQ ID NO: 56 - protein, 13 aa, Homo sapiens
VLQENSSDYQSNL

SEQ ID NO: 57 - protein, 10 aa, Homo sapiens
TLYPGRFDYV

SEQ ID NO: 58 - protein, 11 aa, Homo sapiens
HLLGEGAFAQV

SEQ ID NO: 59 - protein, 11 aa, Homo sapiens
ALADGIKSFLL

SEQ ID NO: 60 - protein, 10 aa, Homo sapiens
YLFSQGLQGL

SEQ ID NO: 61 - protein, 9 aa, Homo sapiens
ALYPKEITL

SEQ ID NO: 62 - protein, 9 aa, Homo sapiens
SLVENIHVL

SEQ ID NO: 63 - protein, 9 aa, Homo sapiens
KLLPMVIQL

SEQ ID NO: 64 - protein, 10 aa, Homo sapiens
SLYAGSNNQV

SEQ ID NO: 65 - protein, 9 aa, Homo sapiens
SLSEKSPEV

SEQ ID NO: 66 - protein, 10 aa, Homo sapiens
AMFPDTIPRV

SEQ ID NO: 67 - protein, 9 aa, Homo sapiens
FLIENLLAA

SEQ ID NO: 68 - protein, 9 aa, Homo sapiens
QLMNLIRSV

SEQ ID NO: 69 - protein, 10 aa, Homo sapiens
LKVLKADVVL

SEQ ID NO: 70 - protein, 9 aa, Homo sapiens
GLTEKTVLV

SEQ ID NO: 71 - protein, 9 aa, Homo sapiens
HMSGKLTNV

SEQ ID NO: 72 - protein, 9 aa, Homo sapiens
VLSTRVTNV

SEQ ID NO: 73 - protein, 8 aa, Homo sapiens
SVPKTLGV

SEQ ID NO: 74 - protein, 9 aa, Homo sapiens
GLAFLPASV

SEQ ID NO: 75 - protein, 9 aa, Homo sapiens
ALLDGALQL

SEQ ID NO: 76 - protein, 9 aa, Homo sapiens
FTAEFLEKV

SEQ ID NO: 77 - protein, 9 aa, Homo sapiens
ALYGNVQQV

SEQ ID NO: 78 - protein, 9 aa, Homo sapiens
LFQSRIAGV

SEQ ID NO: 79 - protein, 10 aa, Homo sapiens
TVLEEIGNRV

SEQ ID NO: 80 - protein, 9 aa, Homo sapiens
VLTGQVHEL

SEQ ID NO: 81 - protein, 9 aa, Homo sapiens
ILAEEPIYI

SEQ ID NO: 82 - protein, 11 aa, Homo sapiens
ILAEEPIYIRV

SEQ ID NO: 83 - protein, 9 aa, Homo sapiens
GLLENSPHL

SEQ ID NO: 84 - protein, 9 aa, Homo sapiens
FLLEREQLL

SEQ ID NO: 85 - protein, 10 aa, Homo sapiens
KLLDKPEQFL

SEQ ID NO: 86 - protein, 9 aa, Homo sapiens
SLFSNIESV

SEQ ID NO: 87 - protein, 9 aa, Homo sapiens
KLLSLLEEA

SEQ ID NO: 88 - protein, 10 aa, Homo sapiens
LLLPLELSLA

SEQ ID NO: 89 - protein, 9 aa, Homo sapiens
SLAETIFIV

SEQ ID NO: 90 - protein, 11 aa, Homo sapiens
AILNVDEKNQV

SEQ ID NO: 91 - protein, 9 aa, Homo sapiens
LLPSIFLMV

SEQ ID NO: 92 - protein, 9 aa, Homo sapiens
RLFEEVLGV

SEQ ID NO: 93 - protein, 9 aa, Homo sapiens
RLYGYFHDA

SEQ ID NO: 94 - protein, 9 aa, Homo sapiens
YLDEVAFML

SEQ ID NO: 95 - protein, 11 aa, Homo sapiens
KLIDEDEPLFL

SEQ ID NO: 96 - protein, 9 aa, Homo sapiens
ALDTTRHEL

SEQ ID NO: 97 - protein, 9 aa, Homo sapiens
KLFEKSTGL

SEQ ID NO: 98 - protein, 9 aa, Homo sapiens
FVQEKIPEL

SEQ ID NO: 99 - protein, 10 aa, Homo sapiens
TLFGIQLTEA

SEQ ID NO: 100 - protein, 9 aa, Homo sapiens
ALQSFEFRV

SEQ ID NO: 101 - protein, 11 aa, Homo sapiens
SLLEVNEASSV

SEQ ID NO: 102 - protein, 10 aa, Homo sapiens
GLYPVTLVGV

SEQ ID NO: 103 - protein, 9 aa, Homo sapiens
YLADTVQKL

SEQ ID NO: 104 - protein, 12 aa, Homo sapiens
DLPTQEPALGTT

SEQ ID NO: 105 - protein, 9 aa, Homo sapiens
AMLASQTEA

SEQ ID NO: 106 - protein, 10 aa, Homo sapiens
VLLGSVVIFA

SEQ ID NO: 107 - protein, 11 aa, Homo sapiens
RVLPGQAVTGV

SEQ ID NO: 108 - protein, 11 aa, Homo sapiens
FIANLPPELKA

SEQ ID NO: 109 - protein, 9 aa, Homo sapiens
ILGSFELQL

SEQ ID NO: 110 - protein, 9 aa, Homo sapiens
QIQGQVSEV

SEQ ID NO: 111 - protein, 10 aa, Homo sapiens
AQLEGKLVSI

SEQ ID NO: 112 - protein, 9 aa, Homo sapiens
ILAQDVAQL

SEQ ID NO: 113 - protein, 9 aa, Homo sapiens
FLFLKEVKV

SEQ ID NO: 114 - protein, 10 aa, Homo sapiens
LLFPSDVQTL

SEQ ID NO: 115 - protein, 9 aa, Homo sapiens
ILHGEVNKV

SEQ ID NO: 116 - protein, 9 aa, Homo sapiens
ALLSSVAEA

SEQ ID NO: 117 - protein, 9 aa, Homo sapiens
TLLEGISRA

SEQ ID NO: 118 - protein, 10 aa, Homo sapiens
IAYNPNGNAL

SEQ ID NO: 119 - protein, 9 aa, Homo sapiens
SLIEESEEL

SEQ ID NO: 120 - protein, 11 aa, Homo sapiens
LQLSPLKGLSL

SEQ ID NO: 121 - protein, 9 aa, Homo sapiens
ALYVQAPTV

SEQ ID NO: 122 - protein, 9 aa, Homo sapiens
SIIDTELKV

SEQ ID NO: 123 - protein, 11 aa, Homo sapiens
QTAPEEAFIKL

SEQ ID NO: 124 - protein, 9 aa, Homo sapiens
ALLLRLFTI

SEQ ID NO: 125 - protein, 9 aa, Homo sapiens
AALEVLAEV

SEQ ID NO: 126 - protein, 9 aa, Homo sapiens
QLREAFEQL

SEQ ID NO: 127 - protein, 11 aa, Homo sapiens
IMKATGLGIQL

SEQ ID NO: 128 - protein, 9 aa, Homo sapiens
SILTNISEV

SEQ ID NO: 129 - protein, 9 aa, Homo sapiens
KMASKVTQV

SEQ ID NO: 130 - protein, 9 aa, Homo sapiens
QLYGSAITL

SEQ ID NO: 131 - protein, 9 aa, Homo sapiens
SLYPHFTLL

SEQ ID NO: 132 - protein, 9 aa, Homo sapiens
ALLNNVIEV

SEQ ID NO: 133 - protein, 9 aa, Homo sapiens
FLDGRPLTL

SEQ ID NO: 134 - protein, 9 aa, Homo sapiens
SLYKSFLQL

SEQ ID NO: 135 - protein, 9 aa, Homo sapiens
HLDTVKIEV

SEQ ID NO: 136 - protein, 9 aa, Homo sapiens
LLWDAPAKC

SEQ ID NO: 137 - protein, 10 aa, Homo sapiens
KLIYKDLVSV

SEQ ID NO: 138 - protein, 9 aa, Homo sapiens
GIINKLVTV

SEQ ID NO: 139 - protein, 9 aa, Homo sapiens
IILENIQSL

SEQ ID NO: 140 - protein, 9 aa, Homo sapiens
FLDSQITTV

SEQ ID NO: 141 - protein, 9 aa, Homo sapiens
NIDINNNEL

SEQ ID NO: 142 - protein, 9 aa, Homo sapiens
LLDAAHASI

SEQ ID NO: 143 - protein, 9 aa, Homo sapiens
MLWESIMRV

SEQ ID NO: 144 - protein, 9 aa, Homo sapiens
FLISQTPLL

SEQ ID NO: 145 - protein, 9 aa, Homo sapiens
ALEEKLENV

SEQ ID NO: 146 - protein, 9 aa, Homo sapiens
VVAAHLAGA

SEQ ID NO: 147 - protein, 9 aa, Homo sapiens
GLLSALENV

SEQ ID NO: 148 - protein, 9 aa, Homo sapiens
YLILSSHQL

SEQ ID NO: 149 - protein, 10 aa, Homo sapiens
NMADGQLHQV

SEQ ID NO: 150 - protein, 9 aa, Homo sapiens
VLLDMVHSL

SEQ ID NO: 151 - protein, 9 aa, Homo sapiens
DISKRIQSL

SEQ ID NO: 152 - protein, 9 aa, Homo sapiens
ILVTSIFFL

SEQ ID NO: 153 - protein, 9 aa, Homo sapiens
KLVELEHTL

SEQ ID NO: 154 - protein, 9 aa, Homo sapiens
AIIKEIQTV

SEQ ID NO: 155 - protein, 9 aa, Homo sapiens
TLDSYLKAV

SEQ ID NO: 156 - protein, 9 aa, Homo sapiens
VILTSSPFL

SEQ ID NO: 157 - protein, 9 aa, Homo sapiens
ILQDGQFLV

SEQ ID NO: 158 - protein, 9 aa, Homo sapiens
YLDPLWHQL

SEQ ID NO: 159 - protein, 9 aa, Homo sapiens
QLGPVPVTI

SEQ ID NO: 160 - protein, 9 aa, Homo sapiens
TLQEWLTEV

SEQ ID NO: 161 - protein, 9 aa, Homo sapiens
NLLDENVCL

SEQ ID NO: 162 - protein, 10 aa, Homo sapiens
GLLGNLLTSL

SEQ ID NO: 163 - protein, 9 aa, Homo sapiens
GLEERLYTA

SEQ ID NO: 164 - protein, 9 aa, Homo sapiens
MLIIRVPSV

SEQ ID NO: 165 - protein, 9 aa, Homo sapiens
SLLDYEVSI

SEQ ID NO: 166 - protein, 9 aa, Homo sapiens
LLGDSSFFL

SEQ ID NO: 167 - protein, 11 aa, Homo sapiens
LVVDEGSLVSV

SEQ ID NO: 168 - protein, 10 aa, Homo sapiens
VIFEGEPMYL

SEQ ID NO: 169 - protein, 9 aa, Homo sapiens
ALADLSVAV

SEQ ID NO: 170 - protein, 9 aa, Homo sapiens
FIAAVVEKV

SEQ ID NO: 171 - protein, 9 aa, Homo sapiens
LLLLDVPTA

SEQ ID NO: 172 - protein, 12 aa, Homo sapiens
SLYLQMNSLRTE

SEQ ID NO: 173 - protein, 9 aa, Homo sapiens
RLIDIYKNV

SEQ ID NO: 174 - protein, 10 aa, Homo sapiens
ALYSGDLHAA

SEQ ID NO: 175 - protein, 9 aa, Homo sapiens
SLLDLVQSL

SEQ ID NO: 176 - protein, 9 aa, Homo sapiens
VQSGLRILL

SEQ ID NO: 177 - protein, 9 aa, Homo sapiens
ALINVLNAL

SEQ ID NO: 178 - protein, 9 aa, Homo sapiens
SLVSWQLLL

SEQ ID NO: 179 - protein, 9 aa, Homo sapiens
TLGEIIKGV

SEQ ID NO: 180 - protein, 9 aa, Homo sapiens
RLYEEEIRI

SEQ ID NO: 181 - protein, 9 aa, Homo sapiens
LLWAPTAQA

SEQ ID NO: 182 - protein, 10 aa, Homo sapiens
GLQDGFQITV

SEQ ID NO: 183 - protein, 9 aa, Homo sapiens
ALSYILPYL

SEQ ID NO: 184 - protein, 9 aa, Homo sapiens
ALDSTIAHL

SEQ ID NO: 185 - protein, 10 aa, Homo sapiens
TLYQGLPAEV

SEQ ID NO: 186 - protein, 9 aa, Homo sapiens
SLLSLESRL

SEQ ID NO: 187 - protein, 9 aa, Homo sapiens
SILKEDPFL

SEQ ID NO: 188 - protein, 9 aa, Homo sapiens
VLGEEQEGV

SEQ ID NO: 189 - protein, 9 aa, Homo sapiens
MAVSDLLIL

SEQ ID NO: 190 - protein, 9 aa, Homo sapiens
SLSTELFKV

SEQ ID NO: 191 - protein, 9 aa, Homo sapiens
AAIEIFEKV

SEQ ID NO: 192 - protein, 11 aa, Homo sapiens
TLLPSSGLVTL

SEQ ID NO: 193 - protein, 9 aa, Homo sapiens
ALFHMNILL

SEQ ID NO: 194 - protein, 9 aa, Homo sapiens
KLLEEVQLL

SEQ ID NO: 195 - protein, 9 aa, Homo sapiens
VIIQNLPAL

SEQ ID NO: 196 - protein, 9 aa, Homo sapiens
TLHQWIYYL

SEQ ID NO: 197 - protein, 10 aa, Homo sapiens
LGGPTSLLHV

SEQ ID NO: 198 - protein, 9 aa, Homo sapiens
ILTNKVVSV

SEQ ID NO: 199 - protein, 9 aa, Homo sapiens
SVADLAHVL

SEQ ID NO: 200 - protein, 10 aa, Homo sapiens
IMPTFDLTKV

SEQ ID NO: 201 - protein, 9 aa, Homo sapiens
LLFSLLCEA

SEQ ID NO: 202 - protein, 9 aa, Homo sapiens
ALAKDELSL

SEQ ID NO: 203 - protein, 9 aa, Homo sapiens
FLFVDPELV

SEQ ID NO: 204 - protein, 11 aa, Homo sapiens
SEWGSPHAAVP

SEQ ID NO: 205 - protein, 9 aa, Homo sapiens
LAFGYDDEL

SEQ ID NO: 206 - protein, 9 aa, Homo sapiens
GLDAFRIFL

SEQ ID NO: 207 - protein, 9 aa, Homo sapiens
KLFETVEEL

SEQ ID NO: 208 - protein, 9 aa, Homo sapiens
HLNNDRNPL

SEQ ID NO: 209 - protein, 10 aa, Homo sapiens
VLQTEELVAN

SEQ ID NO: 210 - protein, 9 aa, Homo sapiens
GLAGDNIYL

SEQ ID NO: 211 - protein, 9 aa, Homo sapiens
LLTTVLINA

SEQ ID NO: 212 - protein, 9 aa, Homo sapiens
MTLSEIHAV

SEQ ID NO: 213 - protein, 10 aa, Homo sapiens
ILAVDGVLSV

SEQ ID NO: 214 - protein, 9 aa, Homo sapiens
ALFETLIQL

SEQ ID NO: 215 - protein, 9 aa, Homo sapiens
QIADIVTSV

SEQ ID NO: 216 - protein, 9 aa, Homo sapiens
ALSTVTPRI

SEQ ID NO: 217 - protein, 9 aa, Homo sapiens
LLWPSSVPA

SEQ ID NO: 218 - protein, 9 aa, Homo sapiens
SLTGANITV

SEQ ID NO: 219 - protein, 9 aa, Homo sapiens
GVVPTIQKV

SEQ ID NO: 220 - protein, 9 aa, Homo sapiens
ALSELERVL

SEQ ID NO: 221 - protein, 9 aa, Homo sapiens
IMLNSVEEI

SEQ ID NO: 222 - protein, 9 aa, Homo sapiens
LLTGVFAQL

SEQ ID NO: 223 - protein, 9 aa, Homo sapiens
ALHPVQFYL

SEQ ID NO: 224 - protein, 13 aa, Homo sapiens
LLFDWSGTGRADA

SEQ ID NO: 225 - protein, 10 aa, Homo sapiens
FLPQPVPLSV

SEQ ID NO: 226 - protein, 9 aa, Homo sapiens
SLAGNLQEL

SEQ ID NO: 227 - protein, 9 aa, Homo sapiens
SEMEELPSV

SEQ ID NO: 228 - protein, 12 aa, Homo sapiens
SLLELDGINLRL

SEQ ID NO: 229 - protein, 9 aa, Homo sapiens
YLYELEHAL

SEQ ID NO: 230 - protein, 9 aa, Homo sapiens
KLLNMIFSI

SEQ ID NO: 231 - protein, 9 aa, Homo sapiens
LLDDIFIRL

SEQ ID NO: 232 - protein, 9 aa, Homo sapiens
LVVGGIATV

SEQ ID NO: 233 - protein, 9 aa, Homo sapiens
SLFESLEYL

SEQ ID NO: 234 - protein, 10 aa, Homo sapiens
VLLNEILEQV

SEQ ID NO: 235 - protein, 9 aa, Homo sapiens
SLLNQPKAV

SEQ ID NO: 236 - protein, 9 aa, Homo sapiens
KMSELQTYV

SEQ ID NO: 237 - protein, 11 aa, Homo sapiens
ALLEQTGDMSL

SEQ ID NO: 238 - protein, 9 aa, Homo sapiens
HLQEKLQSL

SEQ ID NO: 239 - protein, 11 aa, Homo sapiens
VIIKGLEEITV

SEQ ID NO: 240 - protein, 9 aa, Homo sapiens
SVQENIQQK

SEQ ID NO: 241 - protein, 9 aa, Homo sapiens
KQFEGTVEI

SEQ ID NO: 242 - protein, 9 aa, Homo sapiens
KLQEEIPVL

SEQ ID NO: 243 - protein, 9 aa, Homo sapiens
GLAEFQENV

SEQ ID NO: 244 - protein, 9 aa, Homo sapiens
NVAEIVIHI

SEQ ID NO: 245 - protein, 9 aa, Homo sapiens
ALLEEEEGV

SEQ ID NO: 246 - protein, 9 aa, Homo sapiens
ALAGIVTNV

SEQ ID NO: 247 - protein, 12 aa, Homo sapiens
NLLIDDKGTIKL

SEQ ID NO: 248 - protein, 10 aa, Homo sapiens
VLMQDSRLYL

SEQ ID NO: 249 - protein, 9 aa, Homo sapiens
YLYQILQGI

SEQ ID NO: 250 - protein, 9 aa, Homo sapiens
LMQDSRLYL

SEQ ID NO: 251 - protein, 9 aa, Homo sapiens
LLWGNLPEI

SEQ ID NO: 252 - protein, 9 aa, Homo sapiens
SLMEKNQSL

SEQ ID NO: 253 - protein, 9 aa, Homo sapiens
KLLAVIHEL

SEQ ID NO: 254 - protein, 10 aa, Homo sapiens
ALGDKFLLRV

SEQ ID NO: 255 - protein, 11 aa, Homo sapiens
FLMKNSDLYGA

SEQ ID NO: 256 - protein, 9 aa, Homo sapiens
FLNDIFERI

SEQ ID NO: 257 - protein, 10 aa, Homo sapiens
KLIDHQGLYL

SEQ ID NO: 258 - protein, 9 aa, Homo sapiens
QLVQRVASV

SEQ ID NO: 259 - protein, 12 aa, Homo sapiens
GPGIFPPPPPQP

SEQ ID NO: 260 - protein, 9 aa, Homo sapiens
ALNESLVEC

SEQ ID NO: 261 - protein, 9 aa, Homo sapiens
GLAALAVHL

SEQ ID NO: 262 - protein, 9 aa, Homo sapiens
LLLEAVWHL

SEQ ID NO: 263 - protein, 9 aa, Homo sapiens
SIIEYLPTL

SEQ ID NO: 264 - protein, 9 aa, Homo sapiens
TLHDQVHLL

SEQ ID NO: 265 - protein, 11 aa, Homo sapiens
FLLDKPQDLSI

SEQ ID NO: 266 - protein, 9 aa, Homo sapiens
FLLDKPQDL

SEQ ID NO: 267 - protein, 10 aa, Homo sapiens
YLLDMPLWYL

SEQ ID NO: 268 - protein, 9 aa, Homo sapiens
SLDKDIVAL

SEQ ID NO: 269 - protein, 9 aa, Homo sapiens
GLLDCPIFL

SEQ ID NO: 270 - protein, 9 aa, Homo sapiens
TLLTFFHEL

SEQ ID NO: 271 - protein, 9 aa, Homo sapiens
VLIEYNFSI

SEQ ID NO: 272 - protein, 10 aa, Homo sapiens
FVMEGEPPKL

SEQ ID NO: 273 - protein, 9 aa, Homo sapiens
SLNKQIETV

SEQ ID NO: 274 - protein, 11 aa, Homo sapiens
TLYNPERTITV

SEQ ID NO: 275 - protein, 9 aa, Homo sapiens
AVPPPPSSV

SEQ ID NO: 276 - protein, 9 aa, Homo sapiens
RMPTVLQCV

SEQ ID NO: 277 - protein, 9 aa, Homo sapiens
KLQEELNKV

SEQ ID NO: 278 - protein, 9 aa, Homo sapiens
VLEDKVLSV

SEQ ID NO: 279 - protein, 11 aa, Homo sapiens
VLMDEGAVLTL

SEQ ID NO: 280 - protein, 9 aa, Homo sapiens
HLWGHALFL

SEQ ID NO: 281 - protein, 12 aa, Homo sapiens
LLLESDPKVYSL

SEQ ID NO: 282 - protein, 9 aa, Homo sapiens
SLYALHVKA

SEQ ID NO: 283 - protein, 9 aa, Homo sapiens
ALSELLQQV

SEQ ID NO: 284 - protein, 11 aa, Homo sapiens
KLMDPGSLPPL

SEQ ID NO: 285 - protein, 9 aa, Homo sapiens
MLLDTVQKV

SEQ ID NO: 286 - protein, 9 aa, Homo sapiens
FLTEMVHFI

SEQ ID NO: 287 - protein, 9 aa, Homo sapiens
KIQEILTQV

SEQ ID NO: 288 - protein, 9 aa, Homo sapiens
SLYKGLLSV

SEQ ID NO: 289 - protein, 10 aa, Homo sapiens
ELAGIGILTV

SEQ ID NO: 290 - protein, 9 aa, Homo sapiens
YLLPAIVHI